European Patent Specification EP 3 660 052 B1, published September 3, 2025. Title: Antibody specifically binding to PAUF and use thereof. Applicant: Dong-A University Research Foundation For Industry-Academy Cooperation Prestige BioPharma Pte. Ltd. The sequence listing filed with the application follows.

SEQUENCE LISTING (38 sequences)

SEQ ID NO: 1 - protein, 8 aa, Artificial Sequence
  VH-CDR1 of 2H2, 20C5 and hPMAb22
GFNIKDYY

SEQ ID NO: 2 - protein, 8 aa, Artificial Sequence
  VH-CDR2 of 2H2, 20C5 and hPMAb22
IDPENGNT

SEQ ID NO: 3 - protein, 13 aa, Artificial Sequence
  VH-CDR3 of 2H2 and hPMAb22
ARRAITTATAWFA

SEQ ID NO: 4 - protein, 14 aa, Artificial Sequence
  VH-CDR3 of 2H2 and hPMAb22
ARRAITTATAWFAY

SEQ ID NO: 5 - protein, 12 aa, Artificial Sequence
  VL-CDR1 of 2H2, 20C5 and hPMAb22
QSLLNSRTRKNY

SEQ ID NO: 6 - protein, 3 aa, Artificial Sequence
  VL-CDR2 of 2H2, 20C5 and hPMAb22
WAS

SEQ ID NO: 7 - protein, 7 aa, Artificial Sequence
  VL-CDR3 of 2H2 and hPMAb22
KQSYNLY

SEQ ID NO: 8 - protein, 25 aa, Artificial Sequence
  VH-FR1 of 2H2
QVQLKQSGAELVRPGALVKLSCKAS

SEQ ID NO: 9 - protein, 17 aa, Artificial Sequence
  VH-FR2 of 2H2 and 20C5
MHWVKQRPEQGLEWIGW

SEQ ID NO: 10 - protein, 38 aa, Artificial Sequence
  VH-FR3 of 2H2
IYDPKFQGKASITADTSSNTAYLQLSSLTSEDTAVYYC

SEQ ID NO: 11 - protein, 12 aa, Artificial Sequence
  VH-FR4 of 2H2
YWGQGTLVTVSA

SEQ ID NO: 12 - protein, 11 aa, Artificial Sequence
  VH-FR4 of 2H2
WGQGTLVTVSA

SEQ ID NO: 13 - protein, 26 aa, Artificial Sequence
  VL-FR1 of 2H2
DIVMTQSPSSLAVSAGEKVTMSCKSS

SEQ ID NO: 14 - protein, 17 aa, Artificial Sequence
  VL-FR2 of 2H2 and 20C5
LAWYQQKPGQSPKLLIY

SEQ ID NO: 15 - protein, 36 aa, Artificial Sequence
  VL-FR3 of 2H2 and 20C5
TRESGVPDRFTGSGSGTDFTLTISSVQAEDLAVYYC

SEQ ID NO: 16 - protein, 11 aa, Artificial Sequence
  VL-FR4 of 2H2
TFGAGTKLELK

SEQ ID NO: 17 - protein, 121 aa, Artificial Sequence
  VH of 2H2
QVQLKQSGAELVRPGALVKLSCKASGFNIKDYYMHWVKQRPEQGLEWIGWIDPENGNTIYDPKFQGKASITADTSSNTAYLQLSSLTSEDTAVYYCARRAITTATAWFAYWGQGTLVTVSA

SEQ ID NO: 18 - protein, 112 aa, Artificial Sequence
  VL of 2H2
DIVMTQSPSSLAVSAGEKVTMSCKSSQSLLNSRTRKNYLAWYQQKPGQSPKLLIYWASTRESGVPDRFTGSGSGTDFTLTISSVQAEDLAVYYCKQSYNLYTFGAGTKLELK

SEQ ID NO: 19 - protein, 25 aa, Artificial Sequence [sequence omitted]

SEQ ID NO: 20 - protein, 17 aa, Artificial Sequence
  VH-FR2 of hPMAb22
MHWVRQAPGQGLEWMGW

SEQ ID NO: 21 - protein, 38 aa, Artificial Sequence
  VH-FR3 of hPMAb22
NYAQKFQGRVTMTRDTSISTAYMELSRLRSDDTAVYYC

SEQ ID NO: 22 - protein, 12 aa, Artificial Sequence
  VH-FR4 of hPMAb22
YWGQGTLVTVSS

SEQ ID NO: 23 - protein, 11 aa, Artificial Sequence
  VH-FR4 of hPMAb22
WGQGTLVTVSS

SEQ ID NO: 24 - protein, 26 aa, Artificial Sequence
  VL-FR1 of hPMAb22
DIVMTQSPDSLAVSLGERATINCKSS

SEQ ID NO: 25 - protein, 17 aa, Artificial Sequence
  VL-FR2 of hPMAb22
LAWYQQKPGQPPKLLIY

SEQ ID NO: 26 - protein, 36 aa, Artificial Sequence
  VL-FR3 of hPMAb22
TRESGVPDRFSGSGSGTDFTLTISSLQAEDVAVYYC

SEQ ID NO: 27 - protein, 11 aa, Artificial Sequence
  VL-FR4 of hPMAb22
TFGQGTKVEIK

SEQ ID NO: 28 - protein, 121 aa, Artificial Sequence
  VH of hPMAb22
QVQLVQSGAEVKKPGASVKVSCKASGFNIKDYYMHWVRQAPGQGLEWMGWIDPENGNTNYAQKFQGRVTMTRDTSISTAYMELSRLRSDDTAVYYCARRAITTATAWFAYWGQGTLVTVSS

SEQ ID NO: 29 - protein, 112 aa, Artificial Sequence
  VL of hPMAb22
DIVMTQSPDSLAVSLGERATINCKSSQSLLNSRTRKNYLAWYQQKPGQPPKLLIYWASTRESGVPDRFSGSGSGTDFTLTISSLQAEDVAVYYCKQSYNLYTFGQGTKVEIK

SEQ ID NO: 30 - protein, 12 aa, Artificial Sequence
  VH-CDR3 of 20C5
ARRGWLPAWFAY

SEQ ID NO: 31 - protein, 8 aa, Artificial Sequence
  VL-CDR3 of 20C5
KQSYNLYT

SEQ ID NO: 32 - protein, 25 aa, Artificial Sequence
  VH-FR1 of 20C5
QVQLKESGAELVRPGALVKLSCKAS

SEQ ID NO: 33 - protein, 38 aa, Artificial Sequence
  VH-FR3 of 20C5
IYDPKFQGKASLTADTSSNTAYLQLSSLTSEDTAVYYC

SEQ ID NO: 34 - protein, 11 aa, Artificial Sequence
  VH-FR4 of 20C5
WGQGTLVTVSA

SEQ ID NO: 35 - protein, 26 aa, Artificial Sequence
  VL-FR1 of 20C5
DIVMTQSPSSLAVSAGEKVTLSCKSS

SEQ ID NO: 36 - protein, 10 aa, Artificial Sequence
  VL-FR4 of 20C5
FGGGTKLEIK

SEQ ID NO: 37 - protein, 119 aa, Artificial Sequence
  VH of 20C5
QVQLKESGAELVRPGALVKLSCKASGFNIKDYYMHWVKQRPEQGLEWIGWIDPEHGNTIYDPKFQGKASLTADTSSNTAYLQLSSLTSEDTAVYYCARRGWLPAWFAYWGQGTLVTVSA

SEQ ID NO: 38 - protein, 112 aa, Artificial Sequence
  VL of 20C5
DIVMTQSPSSLAVSAGEKVTLSCKSSQSLLNSRTRKNYLAWYQQKPGQSPKLLIYWASTRESGVPDRFTGSGSGTDFTLTISSVQAEDLAVYYCKQSYNLYTFGGGTKLEIK